European Patent Application EP 4 446 422 A2, published October 16, 2024. Title: Verfahren zur Herstellung von wässerigen Lösungen enthaltend L-Psicose. Applicant: Annikki GmbH. Application EP. The sequence listing filed with the application follows.

SEQUENCE LISTING (22 sequences)

SEQ ID NO: 1 - DNA, 840 bp, Millerozyma farinosa
  source 1..840: mol_type = genomic DNA
atgtctcaagctatctcagcaatcaacgaaagagttggcccattgcccactaaagcaccccaactttcaaaaaacgtattagacctcttttccttgaaaggcaaggtagcatcggtgacaggttcatcgaagggaataggctttgctgtcgcagaagcatacgctcaagcaggggctgatgttgctttgtggtacaattcaagtcctgtcgaggataaggtaaaatacttgaaagagacctacggcgtgaaagtcaaagcctacaagtgtaacgtgggaaacagcgaggaggttgagaaaatagtagaccaaattgcagaggacttcggcacaattgacgtttttgttgctaatgcgggcattgcttggagcgaaggtagatctctcgaggttaagggttacgacgcttggcaaaaaattgtcgactacgacttgagcagtgtatactactgtgctaaggcagtgggtaagatcttccaagaaaagggctccggttcgttaatcctcaccgcatccatgtccggacacattgtgaatgttcctcaaatgcaggcaccatacaatgcggccaaggcggctgtgatccatctaggaaaatctttggctgtcgaatgggctccatttgccagggtcaacaccgtttctcctggctatattgccactgatattggtgaatttgtgctgcccgatgagaagaaaaagtggtggtcattgacacccttgggtagagaaggtcttcctcaagaactcactggtgcatacttgtattttgcttctaacgcatcgacctacactactggggctgacttggtcgtagacggtggctacactgtaccataa

SEQ ID NO: 2 - protein, 279 aa, Millerozyma farinosa
MSQAISAINERVGPLPTKAPQLSKNVLDLFSLKGKVASVTGSSKGIGFAVAEAYAQAGADVALWYNSSPVEDKVKYLKETYGVKVKAYKCNVGNSEEVEKIVDQIAEDFGTIDVFVANAGIAWSEGRSLEVKGYDAWQKIVDYDLSSVYYCAKAVGKIFQEKGSGSLILTASMSGHIVNVPQMQAPYNAAKAAVIHLGKSLAVEWAPFARVNTVSPGYIATDIGEFVLPDEKKKWWSLTPLGREGLPQELTGAYLYFASNASTYTTGADLVVDGGYTVP

SEQ ID NO: 3 - DNA, 785 bp, Gluconobacter frateurii
  source 1..785: mol_type = genomic DNA
atgacacagtctcttcagggcaagatcgtcgccattactggcgcggcttcgggcattggcctcgaatgcgcccgctatctcatcgaagctggcgcggtggtctatcttctggaccgtgacgccaaaactctcgaagacaaaacggcagaactcggcagccaggcccatgcgatcatcgtcgatctcttcgactacaaaaccgtagatgctgcggtcgcgcagatcgttgaggagcagggccggatcgatgttttccacgccaacgccggcgcgtatgtgggcggcaatgtctgggaaggggatcccgatagctgggatgcgatgctgcacctgaacatcaatgcagctttccgctcggtccgtgccgtgctgccgcagatgatgaagcaggaaagtggcgatatcgtcatgaccagctcgatcgcgggcatgatccccatcatggccgagccgatctacacggcctcgaaacatgccgtgcaggcattcgtacatacggtgcgccgacaggtcgcgaagtatggaattcgtgtgggtgcaatccagcctggtcctgtagtcacgcctttgctgaaagactgggatcaggcccgtcttgaagccaacatcaaagcgggtgccctgatggaagccaaggaagtcgccgaagccctgatcttcatcctgacacgttcaaagggtgtcatggtgcgggatctggtcgttctgccacataacttcgacgcctaagcttaagcggccgcactcgagcaccaccaccaccaccactgagatccggctgctaa

SEQ ID NO: 4 - protein, 242 aa, Gluconobacter frateurii
MTQSLQGKIVAITGAASGIGLECARYLIEAGAVVYLLDRDAKTLEDKTAELGSQAHAIIVDLFDYKTVDAAVAQIVEEQGRIDVFHANAGAYVGGNVWEGDPDSWDAMLHLNINAAFRSVRAVLPQMMKQESGDIVMTSSIAGMIPIMAEPIYTASKHAVQAFVHTVRRQVAKYGIRVGAIQPGPVVTPLLKDWDQARLEANIKAGALMEAKEVAEALIFILTRSKGVMVRDLVVLPHNFDA

SEQ ID NO: 5 - DNA, 1062 bp, Galactocandida mastotermitis
  source 1..1062: mol_type = genomic DNA
atgagcacaccggaaaatctgagctttgtgctgcagaaaccgtttgatgtgaaatttgaagatcgtccgattccgaaactgagcgatccgtatagcgttaaaattcaggtgaaaaaaaccggcatttgcggtagtgatgttcactatttcacccatggtgcaattggtgattttgttgttaaagcaccgatggttctgggtcatgaaagcagcggtgttgttctggaagttggtagcgaagttaaaagcctgaaagttggtgatcgtgttgcaatggaaccgggtgttccgagccgtcatagtgatgagtataaaagcggtcgttataatctgtgtccgcacatggcatttgcagcaacccctccgtatgatggcaccctgtgtaaatactatattctgccggaagatttctgcgttaaactgccggaacatgttagcctggaagaaggtgcactggttgaaccgctgagcgttgcagttcatagcagcaaactgggtaacattaaaccgggtagccatgttgcaatttatggtgcaggtccggttggtctgctggttgcagcagttgcaagcgcatttggtgcagaaagcgttaccattattgatctggttgaaagccgtctgaatctggcaaaagaactgggtgcaaccgcaaccgttcaggttgattttaaagataccccgaaagaaagcgcagcaaaagttgttgcagcaaataatggcattgcaccggatgttgttattgatgcaagcggtgcagaagcaagcattaattcagccattaatgcaattcgtccgggtggcacctatgttcaggtgggtatgggtaaaccggatgtgagctttccgattgcaaccctgattggtaaagaactgaccgttaaaggtagctttcgttatggttatggtgattatccgctggcagttagcctgctggcaagcggtaaagttaatgtgaaaaaactgatcacccatgaagtgaaattcgaggatgcagcagaagcatttcagctggttcgtgatggtaaagccattaaatgtattatcaacggtccggaataa

SEQ ID NO: 6 - protein, 353 aa, Galactocandida mastotermitis
MSTPENLSFVLQKPFDVKFEDRPIPKLSDPYSVKIQVKKTGICGSDVHYFTHGAIGDFVVKAPMVLGHESSGVVLEVGSEVKSLKVGDRVAMEPGVPSRHSDEYKSGRYNLCPHMAFAATPPYDGTLCKYYILPEDFCVKLPEHVSLEEGALVEPLSVAVHSSKLGNIKPGSHVAIYGAGPVGLLVAAVASAFGAESVTIIDLVESRLNLAKELGATATVQVDFKDTPKESAAKVVAANNGIAPDVVIDASGAEASINSAINAIRPGGTYVQVGMGKPDVSFPIATLIGKELTVKGSFRYGYGDYPLAVSLLASGKVNVKKLITHEVKFEDAAEAFQLVRDGKAIKCIINGPE

SEQ ID NO: 7 - DNA, 1062 bp, Priestia megaterium
  source 1..1062: mol_type = genomic DNA
atgaataacaacctgccgaaaaccatgaaagcagcagttatgcatggcacccgtgaaattagcattgaaaccctgccgattccgcagattgatgaaaatgaagttctgatcaaagttatggccgttggtatttgtggtagcgatctgcactattacacccagggtcgtattggtaaatacaaagtggaaaaaccgtttatcctgggtcatgaatgtagcggtgaagttgttgcaattggtagcgcagttgaacgttttcgtgttggtgatcgtgttgccgttgaaccgggtgttacctgtggtcattgtgaagcatgtaaagagggtcgttataatctgtgtccggatgttcagtttctggcaacccctccggttgatggtgcatttgttcagtatatcaaaatgcgccaggatttcgtttttctgattccgaatagcctgagctatgaagatgcagcactgattgaaccgtttagcgtgggtattcatgcagcaacccgtaccaaactgcagcctggtagcaccattgcaattatgggtatgggtccggttggtctgatggcagttgcagcagcaaaagcatttggtgcaagcaccattattgcaaccgatctggaaccgctgcgtctggaagcagccaaacgtatgggtgcaacccatgttattaacattcgtgaacaggatccgctgaacgagattaaaaacattaccgaaaatgtgggtgttgatgttgcatgggaaaccgcaggtaatccgaaagcactgcagagcagcctgagcagcattcgtcgtggtggtaaactggcaattgttggtctgccgagccagagcgatattccgctggatgttccgtttattgccgataatgaaatcgatatctatggcatctttcgctatgcaaacacctatccgaaaggcatcaaatttctgaccagcggtgcaattgataccaaaaatctggttaccgatcgttatccgctggcaggtacacgtgaagcaatggaacgtgcactgaatttcaaaaacgaatgcctgaaaatcatcgtgtatccgaacgaataa

SEQ ID NO: 8 - protein, 353 aa, Priestia megaterium
MNNNLPKTMKAAVMHGTREISIETLPIPQIDENEVLIKVMAVGICGSDLHYYTQGRIGKYKVEKPFILGHECSGEVVAIGSAVERFRVGDRVAVEPGVTCGHCEACKEGRYNLCPDVQFLATPPVDGAFVQYIKMRQDFVFLIPNSLSYEDAALIEPFSVGIHAATRTKLQPGSTIAIMGMGPVGLMAVAAAKAFGASTIIATDLEPLRLEAAKRMGATHVINIREQDPLNEIKNITENVGVDVAWETAGNPKALQSSLSSIRRGGKLAIVGLPSQSDIPLDVPFIADNEIDIYGIFRYANTYPKGIKFLTSGAIDTKNLVTDRYPLAGTREAMERALNFKNECLKIIVYPNE

SEQ ID NO: 9 - DNA, 729 bp, Kozakia baliensis
  source 1..729: mol_type = genomic DNA
atgacctctcctctccagggtaagatagccgccatcacgggcggggcttcgggcatcggcctcgaatgtgtccgccagatcgccgcaagtggtgccacggtttatattctcgaccgcgaccatcaggcgctcgacaaggcgcgcgaagaattgggcgagcgcgttcataccatcgaggtcgatctcttccgttacgaaacggtcgatcgcgccatcgaaaccatcgtgtccgaacaaggacgcatcgacattctccatgtcaatgcgggcgcgtatatcggcggcaatgtctgggaaggcgatcccgataaatgggacaagatgctgaatctcaacatcaacgccgccttccgttccgcccgcgccgtcatgcccgccatgatgaagcagaaaagcggcgatatcatcatgacaagctcgatcgcaggcatcgtcccgatcccggcggagccgatctacacggcttccaaacatgcggtgcaagccttcgctcacaccatacgccgccagttggccccgttcggcatccgcgtcggcgccatccagcccggcccggtcgtcacgcccttgctcaatgattgggaccccgagcgccttaaagccaatatcgaggctggcgccatgatgcagccttctgacgtcgccgaagccgtggttttcatgctgtcccgccgcaagggaacggtaatccgcgacttggttctgttaccccattctttcgacgtctaa

SEQ ID NO: 10 - protein, 242 aa, Kozakia baliensis
MTSPLQGKIAAITGGASGIGLECVRQIAASGATVYILDRDHQALDKAREELGERVHTIEVDLFRYETVDRAIETIVSEQGRIDILHVNAGAYIGGNVWEGDPDKWDKMLNLNINAAFRSARAVMPAMMKQKSGDIIMTSSIAGIVPIPAEPIYTASKHAVQAFAHTIRRQLAPFGIRVGAIQPGPVVTPLLNDWDPERLKANIEAGAMMQPSDVAEAVVFMLSRRKGTVIRDLVLLPHSFDV

SEQ ID NO: 11 - DNA, 729 bp, Providencia heimbachae
  source 1..729: mol_type = genomic DNA
atggctatatctctcgaaaacaacgtagctgcaattacaggtgccgcttcaggtatcggtctcgaatgtgcacgcacactgatcaaagcaggcgctaaagttgtcctcattgaccgagcagaagatagactaaatcaattggtcgcagaattaggtgaaaatgcaattccattagttatcgatttaatgaaaccagaacaagtcgatggcatgttagcgcgtattatcgaaaaggcaggcagattagatatctttcatgctaatgctggagcttacattggtgggcccgtagccgaaggcgatcccgatgtttgggataaagtcctaaatttaaatgttaatgccgcattccgctgtgttcgcgcagttctaccacactttatcgcacaaaagtcaggcgatattctattcaccagctctatcgctggtatggttcccgtaatttgggagcctatttacacggcatcaaaatttgcggttcaagcattcgttcattctactcgccgtcaggtttctgaacacggtgtccgtgttggtgctgtattacctggtcctgttgttactgcgttattagatgattggccaaaagaaaaacttgaagaagctttagctaacggtagtttaatgcaacccattgaagttgctgaggctgttctattcatgctgacgcgtccaagaaatattacaattcgcgatttagttattttacccaatagtgttgacctctaa

SEQ ID NO: 12 - protein, 242 aa, Providencia heimbachae
MAISLENNVAAITGAASGIGLECARTLIKAGAKVVLIDRAEDRLNQLVAELGENAIPLVIDLMKPEQVDGMLARIIEKAGRLDIFHANAGAYIGGPVAEGDPDVWDKVLNLNVNAAFRCVRAVLPHFIAQKSGDILFTSSIAGMVPVIWEPIYTASKFAVQAFVHSTRRQVSEHGVRVGAVLPGPVVTALLDDWPKEKLEEALANGSLMQPIEVAEAVLFMLTRPRNITIRDLVILPNSVDL

SEQ ID NO: 13 - DNA, 1374 bp, unidentified
  source 1..1374: mol_type = genomic DNA
atgagcaaaattgttatcgtgggtgcaaatcatgcaggcaccgcagcaattaataccattctggataattatggcagcgaaaatgaagtggttgtgtttgatcagaatagcaacattagctttctgggttgtggtatggcactgtggattggtaaacaaattagcggtccgcagggtctgttttatgcagataaagaaagcctggaagcaaaaggtgccaaaatctatatggaaagtccggttaccgccattgattatgatgcaaaacgtgttaccgcactggttaatggtcaagaacatgttgaaagctacgagaaactgattctggcaaccggtagcaccccgattctgcctccgattaaaggtgcagccattaaagaaggtagtcgcgattttgaagcaaccctgaaaaatctgcagttcgtgaaactgtatcagaatgccgaagatgtgattaacaaactgcaggataaaagccagaatctgaatcgtattgcagttgttggtgcaggttatattggtgttgaactggcagaagcatttaaacgtctgggtaaagaagtgattctgattgacgttgttgatacctgtctggcaggttattatgatcaggatctgagcgaaatgatgcgtcagaatctggaagatcatggtatcgaactggcatttggtgaaaccgttaaagcaattgaaggtgatggtaaagtggaacgtattgttaccgataaagcaagccatgatgtggatatggttattctggcagttggttttcgtccgaatacagcactgggtaatgcaaaactgaaaacctttcgtaatggtgcctttctggtggataaaaaacaagaaaccagcatcccggatgtttatgcaattggtgattgtgcaaccgtgtatgataatgccattaacgacaccaactatattgcactggcaagcaatgcactgcgtagcggtattgttgcaggtcataatgcagccggtcataaactggaaagtctgggtgttcagggtagcaatggtatttcaatttttggcctgaatatggttagcaccggtctgacccaagaaaaagccaaacgttttggttataatccggaagttaccgcctttaccgattttcagaaagccagctttatcgagcatgataactatccggttacgctgaaaattgtgtatgacaaagatagccgtctggttctgggtgcacagatggccagcaaagaagatatgagcatgggtattcacatgtttagcctggccattcaagagaaagttaccattgaacgtctggccctgctggattatttctttctgccgcattttaatcagccgtacaactatatgaccaaagcagcactgaaagccaaataa

SEQ ID NO: 14 - protein, 457 aa, unidentified
MSKIVIVGANHAGTAAINTILDNYGSENEVVVFDQNSNISFLGCGMALWIGKQISGPQGLFYADKESLEAKGAKIYMESPVTAIDYDAKRVTALVNGQEHVESYEKLILATGSTPILPPIKGAAIKEGSRDFEATLKNLQFVKLYQNAEDVINKLQDKSQNLNRIAVVGAGYIGVELAEAFKRLGKEVILIDVVDTCLAGYYDQDLSEMMRQNLEDHGIELAFGETVKAIEGDGKVERIVTDKASHDVDMVILAVGFRPNTALGNAKLKTFRNGAFLVDKKQETSIPDVYAIGDCATVYDNAINDTNYIALASNALRSGIVAGHNAAGHKLESLGVQGSNGISIFGLNMVSTGLTQEKAKRFGYNPEVTAFTDFQKASFIEHDNYPVTLKIVYDKDSRLVLGAQMASKEDMSMGIHMFSLAIQEKVTIERLALLDYFFLPHFNQPYNYMTKAALKAK

SEQ ID NO: 15 - DNA, 1014 bp, Geobacillus stearothermophilus
  source 1..1014: mol_type = genomic DNA
atgaaagctgcagttgtggaacaatttaaaaagccgttacaagtgaaagaagtggaaaaacctaagatctcatacggggaagtattagtgcgcatcaaagcgtgtggggtatgccatacagacttgcatgccgcacatggcgactggcctgtaaagcctaaactgcctctcattcctggccatgaaggcgtcggtgtaattgaagaagtaggtcctggggtaacacatttaaaagttggagatcgcgtaggtatcccttggctttattcggcgtgcggtcattgtgactattgcttaagcggacaagaaacattatgcgaacgtcaacaaaacgctggctattccgtcgatggtggttatgctgaatattgccgtgctgcagccgattatgtcgtaaaaattcctgataacttatcgtttgaagaagccgctccaatcttttgcgctggtgtaacaacatataaagcgctcaaagtaacaggcgcaaaaccaggtgaatgggtagccatttacggtatcggcgggcttggacatgtcgcagtccaatacgcaaaggcgatggggttaaacgtcgttgctgtcgatttaggtgatgaaaaacttgagcttgctaaacaacttggtgcagatcttgtcgtcaatccgaaacatgatgatgcagcacaatggataaaagaaaaagtgggcggtgtgcatgcgactgtcgtcacagctgtttcaaaagccgcgttcgaatcagcctacaaatccattcgtcgcggtggtgcttgcgtactcgtcggattaccgccggaagaaatacctattccaattttcgatacagtattaaatggagtaaaaattattggttctatcgttggtacgcgcaaagacttacaagaggcacttcaatttgcagcagaaggaaaagtaaaaacaattgtcgaagtgcaaccgcttgaaaacattaacgacgtattcgatcgtatgttaaaagggcaaattaacggccgcgtcgtgttaaaagtagattaa

SEQ ID NO: 16 - protein, 337 aa, Geobacillus stearothermophilus
MKAAVVEQFKKPLQVKEVEKPKISYGEVLVRIKACGVCHTDLHAAHGDWPVKPKLPLIPGHEGVGVIEEVGPGVTHLKVGDRVGIPWLYSACGHCDYCLSGQETLCERQQNAGYSVDGGYAEYCRAAADYVVKIPDNLSFEEAAPIFCAGVTTYKALKVTGAKPGEWVAIYGIGGLGHVAVQYAKAMGLNVVAVDLGDEKLELAKQLGADLVVNPKHDDAAQWIKEKVGGVHATVVTAVSKAAFESAYKSIRRGGACVLVGLPPEEIPIPIFDTVLNGVKIIGSIVGTRKDLQEALQFAAEGKVKTIVEVQPLENINDVFDRMLKGQINGRVVLKVD

SEQ ID NO: 17 - DNA, 786 bp, Priestia megaterium
  source 1..786: mol_type = genomic DNA
atgtatacagatttaaaagataaagtagttgtaattacaggtggatcaacaggtttaggacgcgcaatggctgttcgtttcggtcaagaagaagcaaaagttgttattaactattacaacaatgaagaagaagctttagatgcgaaaaaagaagtagaagaagcaggcggacaagcaatcatcgttcaaggcgacgtaacaaaagaagaagatgttgtaaaccttgttcaaacagctattaaagaattcggtacattagacgttatgattaataacgctggtgttgaaaacccagttccttctcatgagttatctttagacaactggaataaagttattgatacaaacttaacaggtgcattcttaggaagccgtgaagcaatcaaatattttgttgaaaacgacattaaaggaaacgttattaacatgtctagtgttcatgaaatgattccttggccattatttgttcattacgcagcaagtaaaggcggtatgaaactaatgacggaaacattggctcttgaatatgcgccaaaaggtatccgcgtaaataacattggaccaggtgcgatgaacacaccaattaacgcagagaaatttgcagatcctgtacaacgtgcagacgtagaaagcatgattccaatgggttacatcggtaaaccagaagaagtagcagcagttgcagcattcttagcatcatcacaagcaagctatgtaacaggtattacattatttgctgatggtggtatgacgaaatacccttctttccaagcaggaagaggctaa

SEQ ID NO: 18 - protein, 261 aa, Priestia megaterium
MYTDLKDKVVVITGGSTGLGRAMAVRFGQEEAKVVINYYNNEEEALDAKKEVEEAGGQAIIVQGDVTKEEDVVNLVQTAIKEFGTLDVMINNAGVENPVPSHELSLDNWNKVIDTNLTGAFLGSREAIKYFVENDIKGNVINMSSVHEMIPWPLFVHYAASKGGMKLMTETLALEYAPKGIRVNNIGPGAMNTPINAEKFADPVQRADVESMIPMGYIGKPEEVAAVAAFLASSQASYVTGITLFADGGMTKYPSFQAGRG

SEQ ID NO: 19 - DNA, 1356 bp, Carnobacterium divergens
  source 1..1356: mol_type = genomic DNA
atgaaagtagtagtagtaggctgtacacatgcaggaacagcggcagttaagacgattttaaatgaacatccagatgcatcagtatcagtatatgagcgtaatgacaatgtctcatttctatcttgtgggattgcgttgtatgttggtggagttgtgaaagatcctgcaggtttgttttattcaagtccagaagaacttgcatcaatgggcgcgaaaattaacatggaacacaatgtgaaaaatatagataatgagaataaggtcgtagtaattgagaatttaaaaacaggcgaaacatttgaagaaagctatgataagttggtaatgacaactggatcatggccaattattcctccaattgatggaatcaatagtgaaaatattcttttgtgtaaaaactataaccaagcaaatgaaattattaaagaatcaaaaaatgctaaaaagattgtcattgttggtggtggctatattggaattgaattagttgaggcatttgcagaatctggcaagcaagtgacgctagttgatggattagatcgtattttaaacaaatatttagatgctgaattcacttctgttttagagcatgatttacaagaaagaggcgttacgctagctttaaaccaaaccgtcgagaaatttgttgccaatgaatcaggtgctgtgacagctgtgaaaacaccagttggagaatatgaggctgatttagttattttatgtgttggatttaaaccaaatactgatttgttgaaggataaagtagagatgttgccaaatggtgccatcgtagtggatgaatatatgagaacaagcgatgaagcgatttttgctgctggcgatagttgcgcggttcattataatccaactggaggctctgcgtatattccgttagctacaaatgcagttagaatgggagctttagttgggaaaaatattgtttctccaacagttaaatatcgtggcacgcaagcaacttctggtttatatttatttggttttaatataggttcaaccggattgactgaaaatagcgctcctcattttggcgtagaggttcgttcagtagttgtagaagataattatcgtccagagtttatgccgacaacagagaaagtaacgatgaaattagtttatgaagtaggaacgaatcggattgttggaggtcaaatcatgtcaaaatatgatgtgacacaatctgccaatacgttatctttatgtgttcaaaataaaatgacgattgaggatttggcttatgtagatttcttcttccaacctcactttgatcgtccttggaactatttaaatattttagcgcaagcagctgttgagcaagagcgtaaactagcaaaataa

SEQ ID NO: 20 - protein, 451 aa, Carnobacterium divergens
MKVVVVGCTHAGTAAVKTILNEHPDASVSVYERNDNVSFLSCGIALYVGGVVKDPAGLFYSSPEELASMGAKINMEHNVKNIDNENKVVVIENLKTGETFEESYDKLVMTTGSWPIIPPIDGINSENILLCKNYNQANEIIKESKNAKKIVIVGGGYIGIELVEAFAESGKQVTLVDGLDRILNKYLDAEFTSVLEHDLQERGVTLALNQTVEKFVANESGAVTAVKTPVGEYEADLVILCVGFKPNTDLLKDKVEMLPNGAIVVDEYMRTSDEAIFAAGDSCAVHYNPTGGSAYIPLATNAVRMGALVGKNIVSPTVKYRGTQATSGLYLFGFNIGSTGLTENSAPHFGVEVRSVVVEDNYRPEFMPTTEKVTMKLVYEVGTNRIVGGQIMSKYDVTQSANTLSLCVQNKMTIEDLAYVDFFFQPHFDRPWNYLNILAQAAVEQERKLAK

SEQ ID NO: 21 - DNA, 1356 bp, synthetic construct
  source 1..1356: mol_type = other DNA; note = Variante von SEQ ID Nr. 19
atgaaagtagtagtagtaggctgtacacatgcaggaacagcggcagttaagacgattttaaatgaacatccagatgcatcagtatcagtatatgagcgtaatgacaatgtctcatttctatcttgtgggattgcgttgtatgttggtggagttgtgaaagatcctgcaggtttgttttattcaagtccagaagaacttgcatcaatgggcgcgaaaattaacatggaacacaatgtgaaaaatatagataatgagaataaggtcgtagtaattgagaatttaaaaacaggcgaaacatttgaagaaagctatgataagttggtaatgacaactggatcatggccaattattcctccaattgatggaatcaatagtgaaaatattcttttgtgtaaaaactataaccaagcaaatgaaattattaaagaatcaaaaaatgctaaaaagattgtcattgttggtggtggctatattgcgattgaattagttgaggcatttgcagaatctggcaagcaagtgacgctagttgcgcgtagcgatcgtattttacgtaaatatttagatgctgaattcacttctgttttagagcatgatttacaagaaagaggcgttacgctagctttaaaccaaaccgtcgagaaatttgttgccaatgaatcaggtgctgtgacagctgtgaaaacaccagttggagaatatgaggctgatttagttattttatgtgttggatttaaaccaaatactgatttgttgaaggataaagtagagatgttgccaaatggtgccatcgtagtggatgaatatatgagaacaagcgatgaagcgatttttgctgctggcgatagttgcgcggttcattataatccaactggaggctctgcgtatattccgttagctacaaatgcagttagaatgggagctttagttgggaaaaatattgtttctccaacagttaaatatcgtggcacgcaagcaacttctggtttatatttatttggttttaatataggttcaaccggattgactgaaaatagcgctcctcattttggcgtagaggttcgttcagtagttgtagaagataattatcgtccagagtttatgccgacaacagagaaagtaacgatgaaattagtttatgaagtaggaacgaatcggattgttggaggtcaaatcatgtcaaaatatgatgtgacacaatctgccaatacgttatctttatgtgttcaaaataaaatgacgattgaggatttggcttatgtagatttcttcttccaacctcactttgatcgtccttggaactatttaaatattttagcgcaagcagctgttgagcaagagcgtaaactagcaaaataa

SEQ ID NO: 22 - protein, 451 aa, synthetic construct
  source 1..451: note = Variante von SEQ ID Nr. 20
MKVVVVGCTHAGTAAVKTILNEHPDASVSVYERNDNVSFLSCGIALYVGGVVKDPAGLFYSSPEELASMGAKINMEHNVKNIDNENKVVVIENLKTGETFEESYDKLVMTTGSWPIIPPIDGINSENILLCKNYNQANEIIKESKNAKKIVIVGGGYIAIELVEAFAESGKQVTLVARSDRILRKYLDAEFTSVLEHDLQERGVTLALNQTVEKFVANESGAVTAVKTPVGEYEADLVILCVGFKPNTDLLKDKVEMLPNGAIVVDEYMRTSDEAIFAAGDSCAVHYNPTGGSAYIPLATNAVRMGALVGKNIVSPTVKYRGTQATSGLYLFGFNIGSTGLTENSAPHFGVEVRSVVVEDNYRPEFMPTTEKVTMKLVYEVGTNRIVGGQIMSKYDVTQSANTLSLCVQNKMTIEDLAYVDFFFQPHFDRPWNYLNILAQAAVEQERKLAK